European Patent Application EP 4 759 927 A1, published June 17, 2026. Title: 酯酶突变体及其应用. Applicant: 天津凯莱英生物科技有限公司. Application CN. The sequence listing filed with the application follows.

SEQUENCE LISTING (2 sequences)

SEQ ID NO: 1 - protein, 381 aa, synthetic construct
MQIQGHYELKFEAVRETFAALFDDPQERGAALCIQVGGETVVDLWAGSADKDGQQAWHSDTIANLFSCTKTFTAVTALQLVGEGKLTLDAPVANYWPEFAQAGKQAITLRQLLSHRAGLPAIRELLPAEALYDWQAMVDALAAETPWWTPGTEHGYAVNTYGWLIGELIRRADGRGPGDSIVARTARPLGLDFHVGLADDEFYRVAHIARGKGNAGDAAAQRLLQVTMREPEALSTRAFTNPPAILTSTNKPEWRRMQQPAHNGHGNARSLAGFYAGLLDGSLLESELLDELTREHSLGQDRTLLTQTRFGLGCMLDQPDVANATFGLGARAFGHPGVGGSVGFADPEHDVAFGFVVNTLGPYILMDPRAQKLVRVLASCL

SEQ ID NO: 2 - DNA, 1146 bp, synthetic construct
  source 1..1146: mol_type = other DNA
atgcagatccaaggccactatgagctgaagttcgaggcagtgcgcgagacgttcgcagcgctgttcgacgacccgcaagagcgtggtgctgcactgtgtatccaggtcggtggcgaaaccgtagtcgacctgtgggcaggtagcgcagataaggacggtcagcaagcgtggcatagcgacaccatcgcaaacctgttctcctgcaccaaaaccttcaccgcggttaccgctctgcagctggtgggcgaaggcaaactgaccctggacgcgcctgtggcaaactactggccagaattcgcgcaggcaggtaaacaggctatcactctgcgccagctgctgagccaccgtgccggtctgccagcaatccgtgaactgctgccggctgaagcactgtacgactggcaagcaatggtggatgccctggcagcagaaaccccgtggtggactccgggtactgaacatggttacgccgttaatacctacggctggctgatcggcgaactgatccgtcgtgcggacggtcgtggtcctggtgactctattgtggcccgtactgctcgtccgctgggtctggatttccatgtcggtctggccgatgacgaattctatcgcgttgcgcacattgcgcgtggcaaaggcaacgcgggcgatgctgcggctcagcgtctgctgcaggttactatgcgtgaaccggaagctctgtctacccgtgctttcaccaacccgccggcgattctgacttccacgaacaaaccggaatggcgccgtatgcagcagccggcgcataacggtcacggtaatgctcgctctctggctggtttttacgcgggtctgctggacggtagcctgctggaatctgagctgctggatgaactgacgcgcgaacactccctgggccaggatcgcaccctgctgacccagactcgctttggtctgggttgtatgctggaccagccggatgttgctaatgccacgtttggcctgggcgcgcgtgcgttcggccacccaggcgtgggcggctctgttggcttcgctgatccggaacacgatgttgcgtttggctttgttgtaaacaccctgggtccgtatattctgatggatccgcgtgcccagaaactggtacgtgtactggcctcctgcctgtaa